European Patent Application EP 4 464 720 A2, published November 20, 2024. Title: NON-HUMAN ANIMALS CAPABLE OF DH-DH REARRANGEMENT IN THE IMMUNOGLOBULIN HEAVY CHAIN CODING SEQUENCES. Applicant: Regeneron Pharmaceuticals, Inc. The sequence listing filed with the application follows.

SEQUENCE LISTING (151 sequences)

SEQ ID NO: 1 - DNA, 22 bp, synthetic construct
  misc_feature 1..22: note = hIgHJ2
  source 1..22: mol_type = other DNA
gaggctgtgctactggtacttc

SEQ ID NO: 2 - DNA, 21 bp, synthetic construct
  misc_feature 1..21: note = hIgHJ2
  source 1..21: mol_type = other DNA
ccgtggcaccctggtcactgt

SEQ ID NO: 3 - DNA, 19 bp, synthetic construct
  misc_feature 1..19: note = hIgHJ2
  source 1..19: mol_type = other DNA
tggtgcctggacagagaag

SEQ ID NO: 4 - DNA, 21 bp, synthetic construct
  misc_feature 1..21: note = VI741-42h1
  source 1..21: mol_type = other DNA
tttttgtgcaccccttaatgg

SEQ ID NO: 5 - DNA, 22 bp, synthetic construct
  misc_feature 1..22: note = VI741-42h1
  source 1..22: mol_type = other DNA
atgtggtattacgatttttgga

SEQ ID NO: 6 - DNA, 27 bp, synthetic construct
  misc_feature 1..27: note = VI741-42h1
  source 1..27: mol_type = other DNA
ctctgtgacactgtgggtataataacc

SEQ ID NO: 7 - DNA, 24 bp, synthetic construct
  misc_feature 1..24: note = VI742h2
  source 1..24: mol_type = other DNA
tgtcacagagtccatcaaaaacct

SEQ ID NO: 8 - DNA, 14 bp, synthetic construct
  misc_feature 1..14: note = VI742h2
  source 1..14: mol_type = other DNA
caccaccccctctc

SEQ ID NO: 9 - DNA, 19 bp, synthetic construct
  misc_feature 1..19: note = VI742h2
  source 1..19: mol_type = other DNA
cctgagaccctggcaagct

SEQ ID NO: 10 - DNA, 19 bp, synthetic construct
  misc_feature 1..19: note = Neo
  source 1..19: mol_type = other DNA
ggtggagaggctattcggc

SEQ ID NO: 11 - DNA, 23 bp, synthetic construct
  misc_feature 1..23: note = Neo
  source 1..23: mol_type = other DNA
tgggcacaacagacaatcggctg

SEQ ID NO: 12 - DNA, 17 bp, synthetic construct
  misc_feature 1..17: note = Neo
  source 1..17: mol_type = other DNA
gaacacggcggcatcag

SEQ ID NO: 13 - DNA, 19 bp, synthetic construct
  misc_feature 1..19: note = Jxn DH2-2
  source 1..19: mol_type = other DNA
atggcgcttgcagcgattc

SEQ ID NO: 14 - DNA, 28 bp, synthetic construct
  misc_feature 1..28: note = Jxn DH2-2
  source 1..28: mol_type = other DNA
ccaatactaacgaggaaatgcaaaccca

SEQ ID NO: 15 - DNA, 21 bp, synthetic construct
  misc_feature 1..21: note = Jxn DH2-2
  source 1..21: mol_type = other DNA
accctcactgttgtccttctg

SEQ ID NO: 16 - DNA, 23 bp, synthetic construct
  misc_feature 1..23: note = Jxn DH2-8
  source 1..23: mol_type = other DNA
gcaaacgtccatctgaaggagaa

SEQ ID NO: 17 - DNA, 27 bp, synthetic construct
  misc_feature 1..27: note = Jxn DH2-8
  source 1..27: mol_type = other DNA
caaataaacgatggcaggctacacccg

SEQ ID NO: 18 - DNA, 22 bp, synthetic construct
  misc_feature 1..22: note = Jxn DH2-8
  source 1..22: mol_type = other DNA
gagttgccgaaccgacttattg

SEQ ID NO: 19 - DNA, 23 bp, synthetic construct
  misc_feature 1..23: note = Jxn DH2-15
  source 1..23: mol_type = other DNA
gcaatggtaggttcatgtccatc

SEQ ID NO: 20 - DNA, 20 bp, synthetic construct
  misc_feature 1..20: note = Jxn DH2-15
  source 1..20: mol_type = other DNA
accgccgctggtactccaat

SEQ ID NO: 21 - DNA, 19 bp, synthetic construct
  misc_feature 1..19: note = Jxn DH2-15
  source 1..19: mol_type = other DNA
ccctggctgtctgggtttg

SEQ ID NO: 22 - DNA, 21 bp, synthetic construct
  misc_feature 1..21: note = hIgHJ6
  source 1..21: mol_type = other DNA
cagcagagggttccatgagaa

SEQ ID NO: 23 - DNA, 22 bp, synthetic construct
  misc_feature 1..22: note = hIgHJ6
  source 1..22: mol_type = other DNA
caggacagggccacggacagtc

SEQ ID NO: 24 - DNA, 20 bp, synthetic construct
  misc_feature 1..20: note = hIgHJ6
  source 1..20: mol_type = other DNA
gccacccagagaccttctgt

SEQ ID NO: 25 - DNA, 20 bp, synthetic construct
  misc_feature 1..20: note = hIgH31
  source 1..20: mol_type = other DNA
atcacactcatcccatcccc

SEQ ID NO: 26 - DNA, 29 bp, synthetic construct
  misc_feature 1..29: note = hIgH31
  source 1..29: mol_type = other DNA
cccttccctaagtaccacagagtgggctc

SEQ ID NO: 27 - DNA, 20 bp, synthetic construct
  misc_feature 1..20: note = hIgH31
  source 1..20: mol_type = other DNA
cacagggaagcaggaactgc

SEQ ID NO: 28 - DNA, 17 bp, synthetic construct
  misc_feature 1..17: note = mIgHp2
  source 1..17: mol_type = other DNA
gccatgcaaggccaagc

SEQ ID NO: 29 - DNA, 24 bp, synthetic construct
  misc_feature 1..24: note = mIgHp2
  source 1..24: mol_type = other DNA
ccaggaaaatgctgccagagcctg

SEQ ID NO: 30 - DNA, 24 bp, synthetic construct
  misc_feature 1..24: note = mIgHp2
  source 1..24: mol_type = other DNA
agttcttgagccttagggtgctag

SEQ ID NO: 31 - DNA, 20 bp, synthetic construct
  misc_feature 1..20: note = mADAM6-1
  source 1..20: mol_type = other DNA
ctgagcatggtgtcccatct

SEQ ID NO: 32 - DNA, 24 bp, synthetic construct
  misc_feature 1..24: note = mADAM6-1
  source 1..24: mol_type = other DNA
tgcagataagtgtcatctgggcaa

SEQ ID NO: 33 - DNA, 24 bp, synthetic construct
  misc_feature 1..24: note = mADAM6-1
  source 1..24: mol_type = other DNA
ccagagtactgtagtggctctaag

SEQ ID NO: 34 - DNA, 20 bp, synthetic construct
  misc_feature 1..20: note = hIgk5
  source 1..20: mol_type = other DNA
ccccgtcctcctcctttttc

SEQ ID NO: 35 - DNA, 32 bp, synthetic construct
  misc_feature 1..32: note = hIgk5
  source 1..32: mol_type = other DNA
tcatgtccattaacccatttaccttttgccca

SEQ ID NO: 36 - DNA, 19 bp, synthetic construct
  misc_feature 1..19: note = hIgk5
  source 1..19: mol_type = other DNA
tgcaagtgctgccagcaag

SEQ ID NO: 37 - DNA, 23 bp, synthetic construct
  misc_feature 1..23: note = hIgK21
  source 1..23: mol_type = other DNA
catttggctacatatcaaagccg

SEQ ID NO: 38 - DNA, 27 bp, synthetic construct
  misc_feature 1..27: note = hIgK21
  source 1..27: mol_type = other DNA
cctgagccagggaacagcccactgata

SEQ ID NO: 39 - DNA, 20 bp, synthetic construct
  misc_feature 1..20: note = hIgK21
  source 1..20: mol_type = other DNA
acatggctgaggcagacacc

SEQ ID NO: 40 - DNA, 20 bp, synthetic construct
  misc_feature 1..20: note = mIgKd2
  source 1..20: mol_type = other DNA
gcaaacaaaaaccactggcc

SEQ ID NO: 41 - DNA, 37 bp, synthetic construct
  misc_feature 1..37: note = mIgKd2
  source 1..37: mol_type = other DNA
ctgttcctctaaaactggactccacagtaaatggaaa

SEQ ID NO: 42 - DNA, 19 bp, synthetic construct
  misc_feature 1..19: note = mIgKd2
  source 1..19: mol_type = other DNA
ggccacattccatgggttc

SEQ ID NO: 43 - DNA, 17 bp, synthetic construct
  misc_feature 1..17: note = hyg
  source 1..17: mol_type = other DNA
tgcggccgatcttagcc

SEQ ID NO: 44 - DNA, 21 bp, synthetic construct
  misc_feature 1..21: note = hyg
  source 1..21: mol_type = other DNA
acgagcgggttcggcccattc

SEQ ID NO: 45 - DNA, 18 bp, synthetic construct
  misc_feature 1..18: note = hyg
  source 1..18: mol_type = other DNA
ttgaccgattccttgcgg

SEQ ID NO: 46 - DNA, 20 bp, synthetic construct
  misc_feature 1..20: note = hIgHD-J.1
  source 1..20: mol_type = other DNA
tggcagctgttcaaccatgt

SEQ ID NO: 47 - DNA, 22 bp, synthetic construct
  misc_feature 1..22: note = hIgHD-J.1
  source 1..22: mol_type = other DNA
atccactgtcccagacagcacc

SEQ ID NO: 48 - DNA, 20 bp, synthetic construct
  misc_feature 1..20: note = hIgHD-J.1
  source 1..20: mol_type = other DNA
ggcggtttgtggagtttcct

SEQ ID NO: 49 - DNA, 20 bp, synthetic construct
  misc_feature 1..20: note = hIgHD-J.2
  source 1..20: mol_type = other DNA
tgttgcctccctgcttctag

SEQ ID NO: 50 - DNA, 23 bp, synthetic construct
  misc_feature 1..23: note = hIgHD-J.2
  source 1..23: mol_type = other DNA
cccagaccctcccttgttcctga

SEQ ID NO: 51 - DNA, 18 bp, synthetic construct
  misc_feature 1..18: note = hIgHD-J.2
  source 1..18: mol_type = other DNA
ggcccacgcattgttcag

SEQ ID NO: 52 - DNA, 3263 bp, synthetic construct
  misc_feature 1..3263: note = >p46458 (23-D3-3-12_delJ1-3 donor]
  source 1..3263: mol_type = other DNA
tacgtaccctggccaccgccacccgggcctctctgctgctgggaaaacaagtcagaaagcaagtggatgagaggtggcgtgacagacccagcttcagatctgctctaccggtataacttcgtataatgtatgctatacgaagttatatgcatggcctccgcgccgggttttggcgcctcccgcgggcgcccccctcctcacggcgagcgctgccacgtcagacgaagggcgcagcgagcgtcctgatccttccgcccggacgctcaggacagcggcccgctgctcataagactcggccttagaaccccagtatcagcagaaggacattttaggacgggacttgggtgactctagggcactggttttctttccagagagcggaacaggcgaggaaaagtagtcccttctcggcgattctgcggagggatctccgtggggcggtgaacgccgatgattatataaggacgcgccgggtgtggcacagctagttccgtcgcagccgggatttgggtcgcggttcttgtttgtggatcgctgtgatcgtcacttggtgagtagcgggctgctgggctggccggggctttcgtggccgccgggccgctcggtgggacggaagcgtgtggagagaccgccaagggctgtagtctgggtccgcgagcaaggttgccctgaactgggggttggggggagcgcagcaaaatggcggctgttcccgagtcttgaatggaagacgcttgtgaggcgggctgtgaggtcgttgaaacaaggtggggggcatggtgggcggcaagaacccaaggtcttgaggccttcgctaatgcgggaaagctcttattcgggtgagatgggctggggcaccatctggggaccctgacgtgaagtttgtcactgactggagaactcggtttgtcgtctgttgcgggggcggcagttatggcggtgccgttgggcagtgcacccgtacctttgggagcgcgcgccctcgtcgtgtcgtgacgtcacccgttctgttggcttataatgcagggtggggccacctgccggtaggtgtgcggtaggcttttctccgtcgcaggacgcagggttcgggcctagggtaggctctcctgaatcgacaggcgccggacctctggtgaggggagggataagtgaggcgtcagtttctttggtcggttttatgtacctatcttcttaagtagctgaagctccggttttgaactatgcgctcggggttggcgagtgtgttttgtgaagttttttaggcaccttttgaaatgtaatcatttgggtcaatatgtaattttcagtgttagactagtaaattgtccgctaaattctggccgtttttggcttttttgttagacgtcgagctagcctagattgggaacccgggtctctcgaattgttgacaattaatcatcggcatagtatatcggcatagtataatacgacaaggtgaggaactaaaccatccaccatgattgaacaagatggattgcacgcaggttctccggccgcttgggtggagaggctattcggctatgactgggcacaacagacaatcggctgctctgatgccgccgtgttccggctgtcagcgcaggggcgcccggttctttttgtcaagaccgacctgtccggtgccctgaatgaactgcaggacgaggcagcgcggctatcgtggctggccacgacgggcgttccttgcgcagctgtgctcgacgttgtcactgaagcgggaagggactggctgctattgggcgaagtgccggggcaggatctcctgtcatctcaccttgctcctgccgagaaagtatccatcatggctgatgcaatgcggcggctgcatacgcttgatccggctacctgcccattcgaccaccaagcgaaacatcgcatcgagcgagcacgtactcggatggaagccggtcttgtcgatcaggatgatctggacgaagagcatcaggggctcgcgccagccgaactgttcgccaggctcaaggcgcgcatgcccgacggcgaggatctcgtcgtgacccatggcgatgcctgcttgccgaatatcatggtggaaaatggccgcttttctggattcatcgactgtggccggctgggtgtggcggaccgctatcaggacatagcgttggctacccgtgatattgctgaagagcttggcggcgaatgggctgaccgcttcctcgtgctttacggtatcgccgctcccgattcgcagcgcatcgccttctatcgccttcttgacgagttcttctgaagatccgctgtaagtctgcagaaattgatgatctattaaacaataaagatgtccactaaaatggaagtttttcctgtcatactttgttaagaagggtgagaacagagtacctacattttgaatggaaggattggagctacgggggtgggggtggggtgggattagataaatgcctgctctttactgaaggctctttactattgctttatgataatgtttcatagttggatatcataatttaaacaagcaaaaccaaattaagggccagctcattcctcccactcatgatctatagatctatagatctctcgtgggatcattgtttttctcttgattcccactttgtggttctaagtactgtggtttccaaatgtgtcagtttcatagcctgaagaacgagatcagcagcctctgttccacatacacttcattctcagtattgttttgccaagttctaattccatcagacctcgacctgcagccggcgcgccataacttcgtataatgtatgctatacgaagttatgtcgacctcgagaatttacaaaagaaaaggaaaaacacacttggcagccttcagcactctaatgattcttaacagcagcaaattattggcacaagactccagagtgactggcagggttgagggctggggtctcccacgtgttttggggctaacagcggaagggagagcactggcaaaggtgctgggggcccctggacccgacccgccctggagaccgcagccacatcagcccccagccccacaggccccctaccagccgcagggtttttgtgcaccccttaatggggcctcccacaatgtggtattacgatttttggagtggttattatacccacagtgtcacagagtccatcaaaaaccaagatggctttccttctgcctcctttctctgggcccagcgtcctctgtcctggagctgggagataatgtccgggggctccttggtctgcgctgggccatgtacgta

SEQ ID NO: 53 - DNA, 23 bp, synthetic construct
  misc_feature 1..23: note = DNA recognition site
  source 1..23: mol_type = other DNA
tcagaaagcaagtggatgagagg

SEQ ID NO: 54 - RNA, 42 nt, synthetic construct
  misc_feature 1..42: note = 5' D7.27 gRNA
  source 1..42: mol_type = other RNA
tcagaaagcaagtggatgaggttttagagctatgctgttttg

SEQ ID NO: 55 - DNA, 23 bp, synthetic construct
  misc_feature 1..23: note = DNA recognition site
  source 1..23: mol_type = other DNA
gctccaggacagaggacgctggg

SEQ ID NO: 56 - RNA, 42 nt, synthetic construct
  misc_feature 1..42: note = 3' JH1-3 del gRNA
  source 1..42: mol_type = other RNA
gctccaggacagaggacgctgttttagagctatgctgttttg

SEQ ID NO: 57 - DNA, 19 bp, synthetic construct
  misc_feature 1..19: note = 5' up detect D7-27
  source 1..19: mol_type = other DNA
gtgaacaggtggaaccaac

SEQ ID NO: 58 - DNA, 21 bp, synthetic construct
  misc_feature 1..21: note = 3' ub pro-200
  source 1..21: mol_type = other DNA
ccagtgccctagagtcaccca

SEQ ID NO: 59 - DNA, 21 bp, synthetic construct
  misc_feature 1..21: note = 5' neo detect
  source 1..21: mol_type = other DNA
ctcccactcatgatctataga

SEQ ID NO: 60 - DNA, 20 bp, synthetic construct
  misc_feature 1..20: note = 3' down detect JH1-3 del
  source 1..20: mol_type = other DNA
gtcccagttcccaaagaaag

SEQ ID NO: 61 - DNA, 3263 bp, synthetic construct
  misc_feature 1..3263: note = >p46459 (23-D3-3-12_delJ1-5 donor)
  source 1..3263: mol_type = other DNA
tacgtaccctggccaccgccacccgggcctctctgctgctgggaaaacaagtcagaaagcaagtggatgagaggtggcgtgacagacccagcttcagatctgctctaccggtataacttcgtataatgtatgctatacgaagttatatgcatggcctccgcgccgggttttggcgcctcccgcgggcgcccccctcctcacggcgagcgctgccacgtcagacgaagggcgcagcgagcgtcctgatccttccgcccggacgctcaggacagcggcccgctgctcataagactcggccttagaaccccagtatcagcagaaggacattttaggacgggacttgggtgactctagggcactggttttctttccagagagcggaacaggcgaggaaaagtagtcccttctcggcgattctgcggagggatctccgtggggcggtgaacgccgatgattatataaggacgcgccgggtgtggcacagctagttccgtcgcagccgggatttgggtcgcggttcttgtttgtggatcgctgtgatcgtcacttggtgagtagcgggctgctgggctggccggggctttcgtggccgccgggccgctcggtgggacggaagcgtgtggagagaccgccaagggctgtagtctgggtccgcgagcaaggttgccctgaactgggggttggggggagcgcagcaaaatggcggctgttcccgagtcttgaatggaagacgcttgtgaggcgggctgtgaggtcgttgaaacaaggtggggggcatggtgggcggcaagaacccaaggtcttgaggccttcgctaatgcgggaaagctcttattcgggtgagatgggctggggcaccatctggggaccctgacgtgaagtttgtcactgactggagaactcggtttgtcgtctgttgcgggggcggcagttatggcggtgccgttgggcagtgcacccgtacctttgggagcgcgcgccctcgtcgtgtcgtgacgtcacccgttctgttggcttataatgcagggtggggccacctgccggtaggtgtgcggtaggcttttctccgtcgcaggacgcagggttcgggcctagggtaggctctcctgaatcgacaggcgccggacctctggtgaggggagggataagtgaggcgtcagtttctttggtcggttttatgtacctatcttcttaagtagctgaagctccggttttgaactatgcgctcggggttggcgagtgtgttttgtgaagttttttaggcaccttttgaaatgtaatcatttgggtcaatatgtaattttcagtgttagactagtaaattgtccgctaaattctggccgtttttggcttttttgttagacgtcgagctagcctagattgggaacccgggtctctcgaattgttgacaattaatcatcggcatagtatatcggcatagtataatacgacaaggtgaggaactaaaccatccaccatgattgaacaagatggattgcacgcaggttctccggccgcttgggtggagaggctattcggctatgactgggcacaacagacaatcggctgctctgatgccgccgtgttccggctgtcagcgcaggggcgcccggttctttttgtcaagaccgacctgtccggtgccctgaatgaactgcaggacgaggcagcgcggctatcgtggctggccacgacgggcgttccttgcgcagctgtgctcgacgttgtcactgaagcgggaagggactggctgctattgggcgaagtgccggggcaggatctcctgtcatctcaccttgctcctgccgagaaagtatccatcatggctgatgcaatgcggcggctgcatacgcttgatccggctacctgcccattcgaccaccaagcgaaacatcgcatcgagcgagcacgtactcggatggaagccggtcttgtcgatcaggatgatctggacgaagagcatcaggggctcgcgccagccgaactgttcgccaggctcaaggcgcgcatgcccgacggcgaggatctcgtcgtgacccatggcgatgcctgcttgccgaatatcatggtggaaaatggccgcttttctggattcatcgactgtggccggctgggtgtggcggaccgctatcaggacatagcgttggctacccgtgatattgctgaagagcttggcggcgaatgggctgaccgcttcctcgtgctttacggtatcgccgctcccgattcgcagcgcatcgccttctatcgccttcttgacgagttcttctgaagatccgctgtaagtctgcagaaattgatgatctattaaacaataaagatgtccactaaaatggaagtttttcctgtcatactttgttaagaagggtgagaacagagtacctacattttgaatggaaggattggagctacgggggtgggggtggggtgggattagataaatgcctgctctttactgaaggctctttactattgctttatgataatgtttcatagttggatatcataatttaaacaagcaaaaccaaattaagggccagctcattcctcccactcatgatctatagatctatagatctctcgtgggatcattgtttttctcttgattcccactttgtggttctaagtactgtggtttccaaatgtgtcagtttcatagcctgaagaacgagatcagcagcctctgttccacatacacttcattctcagtattgttttgccaagttctaattccatcagacctcgacctgcagccggcgcgccataacttcgtataatgtatgctatacgaagttatgtcgacctcgagaatttacaaaagaaaaggaaaaacacacttggcagccttcagcactctaatgattcttaacagcagcaaattattggcacaagactccagagtgactggcagggttgagggctggggtctcccacgtgttttggggctaacagcggaagggagagcactggcaaaggtgctgggggcccctggacccgacccgccctggagaccgcagccacatcagcccccagccccacaggccccctaccagccgcagggtttttgtgcaccccttaatggggcctcccacaatgtggtattacgatttttggagtggttattatacccacagtgtcacagagtccatcaaaaacctcctcaccaccccctctctgagtccacttagggagactcagcttgccagggtctcagggtcagagtcttggaggcattttggaggtcaggaaagaaagcctacgta

SEQ ID NO: 62 - DNA, 23 bp, synthetic construct
  misc_feature 1..23: note = DNA recognition site
  source 1..23: mol_type = other DNA
tcagaaagcaagtggatgagagg

SEQ ID NO: 63 - RNA, 42 nt, synthetic construct; identical to SEQ ID NO: 54
  misc_feature 1..42: note = 5' D7.27 crRNA
  source 1..42: mol_type = other RNA

SEQ ID NO: 64 - DNA, 23 bp, synthetic construct
  misc_feature 1..23: note = DNA recognition site
  source 1..23: mol_type = other DNA
ttagggagactcagcttgccagg

SEQ ID NO: 65 - RNA, 42 nt, synthetic construct
  misc_feature 1..42: note = 3' JH1-5 del crRNA
  source 1..42: mol_type = other RNA
ttagggagactcagcttgccgttttagagctatgctgttttg

SEQ ID NO: 66 - DNA, 19 bp, synthetic construct
  misc_feature 1..19: note = 5' up detect D7-27
  source 1..19: mol_type = other DNA
gtgaacaggtggaaccaac

SEQ ID NO: 67 - DNA, 21 bp, synthetic construct
  misc_feature 1..21: note = 3' ub pro-200
  source 1..21: mol_type = other DNA
ccagtgccctagagtcaccca

SEQ ID NO: 68 - DNA, 21 bp, synthetic construct
  misc_feature 1..21: note = 5' neo detect
  source 1..21: mol_type = other DNA
ctcccactcatgatctataga

SEQ ID NO: 69 - DNA, 19 bp, synthetic construct
  misc_feature 1..19: note = 3' down detect JH1-5 del
  source 1..19: mol_type = other DNA
acgcaatcatcacgacagc

SEQ ID NO: 70 - DNA, 3345 bp, synthetic construct
  misc_feature 1..3345: note = >p51816 (12-D2-2-23 donor)
  source 1..3345: mol_type = other DNA
actagtagaagataagctccagacccccaagactgggacctgccttcctgccaccgcgccggcgatgcatccgggtaggggaggcgcttttcccaaggcagtctggagttgacaattaatcatcggcatagtatatcggcatagtataatacgacaaggtgaggaactaaaccatggagaaaaaaatcactggatataccaccgttgatatatcccaatggcatcgtaaagaacattttgaggcatttcagtcagttgctcaatgtacctataaccagaccgttcagctggatattacggcctttttaaagaccgtaaagaaaaataagcacaagttttatccggcctttattcacattcttgcccgcctgatgaatgctcatccggaattccgtatggcaatgaaagacggtgagctggtgatatgggatagtgttcacccttgttacaccgttttccatgagcaaactgaaacgttttcatcgctctggagtgaataccacgacgatttccggcagtttctacacatatattcgcaagatgtggcgtgttacggtgaaaacctggcctatttccctaaagggtttattgagaatatgtttttcgtctcagccaatccctgggtgagtttcaccagttttgatttaaacgtggccaatatggacaacttcttcgcccccgttttcaccatgggcaaatattatacgcaaggcgacaaggtgctgatgccgctggcgattcaggttcatcatgccgtttgtgatggcttccatgtcggcagaatgcttaatgaattacaacagtactgcgatgagtggcagggcggggcgtaaggatcctgccatttcattacctctttctccgcacccgacatagataaagcttatcgataccgtcgacctcgagggggggcccggtacccgccggcgcttgtagctccagacctccgtgcctcccccgaccacttactgttagataggcattgatctaggcacggggcgcgatgttgacacgggccagggagctgttccacaaagatcaaccccaaaccgggaccgcctggcactcgcgccgctgccacttccctctccatttgttcccagcacctctgtgctccctccctcctccctccttcaggggaacagcctgtgcagcccctccctgcaccccacaccctggggaggcccaaccctgcctccagccctttctcccccgctgctcttcctgcccatccagacaaccctggggtcccatccctgcagcctacaccctggtctccacccagacccctgtctctccctccagacacccctcccaggccaaccctgcacacgcaggccctccccttttctgctcccagagcctcaccctctaccctctgtgcctaccccctgcctcctcctgcccacaactcgagctcttcctctcctggggcccctgagccatggcactgaccgtgcactcccacccccacactgcccatgccctcaccttcctcctggacactctgaccccgctcccctcttggacccagccctggtatttccaggacaaaggctcacccaagtcttccccatgcaggcccttgccctcactgcccggttacacggcagcctcctgtgcacagaagcagggagctcagcccttccacaggcagaaggcactgaaagaaatcggcctccagcaccctgatgcacgtccgcctgtgtctctcactgcccgcacctgcagggaggctcggcactccctgtaaagacgagggatccaggcagcaacatcatgggagaatgcagggctcccagacagcccagccctctcgcaggcctctcctgggaagagacctgcagccaccactgaacagccacggagcccgctggatagtaactgagtcagtgaccgacctggagggcaggggagcagtgaaccggagcccagaccatagggacagagaccagccgctgacatcccgagcccctcactggcggccccagaacaccgcgtggaaacagaacagacccacattcccacctggaaaagggcagacactgctgagcccccagcaccagccctgagaaacaccaggcaacggcatcagagggggctcctgagaaagaaaggaggggaggtctccttcaccagcaagtacttcccttgaccaaaaacagggtccacgcaactcccccaggacaaaggaggagccccctgtacagcactgggctcagagtcctctcccacacaccctgagtttcagacaaaaaccccctggaaatcatagtatcagcaggagaactagccagagacagcaagaggggactcagtgactcccgcggggacaggaggattttgtgggggctcgtgtcactgtgaggatattgtagtagtaccagctgctatacccacagtgtgaaaacccacatcctgagagtgacacaaacccctgctgtaaacgcttccacttctggagctgaggggctggggggagcgtctgggaagtagggcctaggggtggccatcaatgcccaaaacgcaccagactcccccccagacatcaccccactggccagtgagcagagtaaacagaaaatgagaagcagctgggaagcttgcacaggccccaaggaaagagctttggcgggtgtgcaagaggggatgcgggcagagcctgagcagggccttttgctgtttctgctttcctgtgcagatagttccataaactggtgttcaagatcgatggctgggagtgagcccaggaggacagtgtgggaagggcacagggaaggagaagcagccgctatcctacactgtcatctttcaagagtttgccctgtgcccacaatgctgcatcatgggatgcttaacagctgatgtagacacagctaaagagagaatcagtgaaatggatttgcagcacagatctgaataaattctccagaatgtggagccacacagaagcaagcacaaggaaagtgcctgatgcaagggcaaagtacagtgtgtaccttcaggctgggcacagacactctgaaaagccttggcaggaactccctgcaacaaagcagagccctgcaggcaatgccagctccagagccctccctgagagcctcatgggcaaagatgtgcacaacaggtgtttctcatagccccaaactgagaatgaagcaaacagccatctgaaggaaaacaggcaaataaacgatggcaggttcatggcgcttgcagcgattcaacagctaaccaatactaacgaggaaatgcaaacccagacagccagaaggacaacagtgagggttacaggtgactctgtggttgagttcatgacaatgctgagtaattggagtaactagt

SEQ ID NO: 71 - DNA, 2484 bp, synthetic construct
  misc_feature 1..2484: note = >p53419 (12-D2-8-23 donor)
  source 1..2484: mol_type = other DNA
actagtcccagtcctctcacaggcctctcctgggaagagacctgaagacgcccagtcgccggcgatgcatccgggtaggggaggcgcttttcccaaggcagtctggagttgacaattaatcatcggcatagtatatcggcatagtataatacgacaaggtgaggaactaaaccatggagaaaaaaatcactggatataccaccgttgatatatcccaatggcatcgtaaagaacattttgaggcatttcagtcagttgctcaatgtacctataaccagaccgttcagctggatattacggcctttttaaagaccgtaaagaaaaataagcacaagttttatccggcctttattcacattcttgcccgcctgatgaatgctcatccggaattccgtatggcaatgaaagacggtgagctggtgatatgggatagtgttcacccttgttacaccgttttccatgagcaaactgaaacgttttcatcgctctggagtgaataccacgacgatttccggcagtttctacacatatattcgcaagatgtggcgtgttacggtgaaaacctggcctatttccctaaagggtttattgagaatatgtttttcgtctcagccaatccctgggtgagtttcaccagttttgatttaaacgtggccaatatggacaacttcttcgcccccgttttcaccatgggcaaatattatacgcaaggcgacaaggtgctgatgccgctggcgattcaggttcatcatgccgtttgtgatggcttccatgtcggcagaatgcttaatgaattacaacagtactgcgatgagtggcagggcggggcgtaaggatcctgccatttcattacctctttctccgcacccgacatagataaagcttatcgataccgtcgacctcgagggggggcccggtacccgccggcgcaacggagtctaacaccaaacctccctggaggccgatgggcgagcaaaatccgacacgtaactacaagtagggcctgatctagtaacggagtcattgccagacctggaggcaggggagcagtgagcccgagcccacaccatagggccagagggcacagcaactgacatcccaagccactcactggtggtcccacaacaccccatggaaagaggacagacccacagtcccacctggaccagggcagagactgctgagacccagcaccagaaccaaccaagaaacaccaggcaacagcatcagagggggctctggcagaacagaggaggggaggtctccttcaccagcaggcgcttcccttgaccgaagacaggatccatgcaactcccccaggacaaaggaggagccccttgttcagcactgggctcagagtcctctccaagacacccagagtttcagacaaaaaccccctggaatgcacagtctcagcaggagagccagccagagccagcaagatggggctcagtgacacccgcagggacaggaggattttgtgggggctcgtgtcactgtgaggatattgtactaatggtgtatgctatacccacagtgtgaaaacccacatcctgagagtgacacaaacccctactgcaaacgcattccacttctggggctgaggggctgggggagcgtctgggaaatagggctcaggggtgtccatcaatgcccaaaacgcaccagactcccctccatacatcacacccaccagccagcgagcagagtaaacagaaaatgagaagcaagctggggaagcttgcacaggccccaaggaaagagctttggcgggtgtgtaagaggggatgcgggcagagcctgagcagggccttttgctgtttctgctttcctgtgcagagagttccataaactggtgttcgagatcaatggctgggagtgagcccaggaggacagcgtgggaagagcacagggaaggaggagcagccgctatcctacactgtcatctttcaaaagtttcccttgtgcccacattgctgcatcatgggatgcttaagagctgatgtagacacagctaaagagagaatcagtgagatggatttgcagcacagatctgaataaattctccagaatgtggagcagcacagaagcaagcacacagaaagtgcctgatgcaaggacaaagttcagtgggcaccttcaggcattgctgctgggcacagacattctgaaaagccctggcaggaactccctgtgacaaagcagaaccctcaggcaatgccagccccagagccctccctgagagcctcatgggcaaagatgtgcacaacaggtgtttctcatagccccaaactgagagcaaagcaaacgtccatctgaaggagaacaggcaaataaacgatggcaggctacacccgtgcatccaataagtcggttcggcaactcaacttcatgaaatgcaaacccagacagccacaagcacaaaagtacagggttataagcgactctggttgagttcatgacaatgctgagtaattgactagt

SEQ ID NO: 72 - DNA, 2321 bp, synthetic construct
  misc_feature 1..2321: note = >p51818 (12-D2-15-23 donor)
  source 1..2321: mol_type = other DNA
actagtgagaccagccgctgacatcccgagctcctcaatggtggccccataacacacgccggcgatgcatccgggtaggggaggcgcttttcccaaggcagtctggagttgacaattaatcatcggcatagtatatcggcatagtataatacgacaaggtgaggaactaaaccatggagaaaaaaatcactggatataccaccgttgatatatcccaatggcatcgtaaagaacattttgaggcatttcagtcagttgctcaatgtacctataaccagaccgttcagctggatattacggcctttttaaagaccgtaaagaaaaataagcacaagttttatccggcctttattcacattcttgcccgcctgatgaatgctcatccggaattccgtatggcaatgaaagacggtgagctggtgatatgggatagtgttcacccttgttacaccgttttccatgagcaaactgaaacgttttcatcgctctggagtgaataccacgacgatttccggcagtttctacacatatattcgcaagatgtggcgtgttacggtgaaaacctggcctatttccctaaagggtttattgagaatatgtttttcgtctcagccaatccctgggtgagtttcaccagttttgatttaaacgtggccaatatggacaacttcttcgcccccgttttcaccatgggcaaatattatacgcaaggcgacaaggtgctgatgccgctggcgattcaggttcatcatgccgtttgtgatggcttccatgtcggcagaatgcttaatgaattacaacagtactgcgatgagtggcagggcggggcgtaaggatcctgccatttcattacctctttctccgcacccgacatagataaagcttatcgataccgtcgacctcgagggggggcccggtacccgccggcgcctaggaaacataacacacccacagccccacctggaacagatagatgcaccaatatctcccagtaagctcaagctcgcggggcagagactgctgagcccccagcaccagccccaagaaacaccaggcaacagtatcagagggggctcccgagaaagagaggaggggagatctccttcaccatcaaatgcttcccttgaccaaaaacagggtccacgcaactcccccaggacaaaggaggagccccctatacagcactgggctcagagtcctctctgagacaccctgagtttcagacaacaacccgctggaatgcacagtctcagcaggagaacagaccaaagccagcaaaagggacctcggtgacaccagtagggacaggaggattttgtgggggctcgtgtcactgtgaggatattgtagtggtggtagctgctactcccacagtgtgaaaacccacatcctgagagtgacacaaacccctactgcaaacacccccactcctggggctgaggggctaggggagcgtctgggaagtagggtccaggggtgtctatcaatgtccaaaatgcaccagactccccgccaaacaccaccccaccagccagcgagcagggtaaacagaaaatgagaggctctgggaagcttgcacaggccccaaggaaagagctttggcgggtgtgcaagaggggatgcaggcagagcctgagcagggccttttgctgtttctgctttcctgtgcagagagttccataaactggtgttcaagatcagtggctgggaatgagcccaggagggcagtctgtgggaagagcacagggaaggaggagcagccgctatcctacactgtcatctttcaaaagtttgccttgtgaccacactattgcatcatgggatgcttaagagctgatgtagacacagctaaagagagaatcagtgagatgaatttgcagcatagatctgaataaactctccagaatgtggagcagtacagaagcaaacacacagaaagtgcctgatgcaaggacaaagttcagtgggcaccttcaggcattgctgctgggcacagacactctgaaaagccctggcaggatctccctgcgacaaagcagaaccctcaggcaatgccagccccagagccctccctgagagcgtcatggggaaagatgtgcagaacagctgattatcatagactcaaactgagaacagagcaaacgtccatctgaagaacagtcaaataagcaatggtaggttcatgtccatctcatcggtcagtaaaaataccgccgctggtactccaatgcaaacccagacagccaggggacaacagtagagggctacaggcggctttgcggttgagttcatgacaatgctgagtaattggagtaactagt

SEQ ID NO: 73 - DNA, 40 bp, synthetic construct
  misc_feature 1..40: note = 1 P51816(D2-2)
  source 1..40: mol_type = other DNA
tgttagataggcattgatctaggcacggggcgcgatgttg

SEQ ID NO: 74 - DNA, 40 bp, synthetic construct
  misc_feature 1..40: note = 2 P51816(D2-2)
  source 1..40: mol_type = other DNA
gcgcttgcagcgattcaacagctaaccaatactaacgagg

SEQ ID NO: 75 - DNA, 40 bp, synthetic construct
  misc_feature 1..40: note = 10 P53419(D2-8)
  source 1..40: mol_type = other DNA
cgagcaaaatccgacacgtaactacaagtagggcctgatc

SEQ ID NO: 76 - DNA, 40 bp, synthetic construct
  misc_feature 1..40: note = 16 P53419(D2-8)
  source 1..40: mol_type = other DNA
ctacacccgtgcatccaataagtcggttcggcaactcaac

SEQ ID NO: 77 - DNA, 40 bp, synthetic construct
  misc_feature 1..40: note = 8 P51818(D2-15)
  source 1..40: mol_type = other DNA
atagatgcaccaatatctcccagtaagctcaagctcgcgg

SEQ ID NO: 78 - DNA, 40 bp, synthetic construct
  misc_feature 1..40: note = 18 P51818(D2-15)
  source 1..40: mol_type = other DNA
tccatctcatcggtcagtaaaaataccgccgctggtactc

SEQ ID NO: 79 - DNA, 20 bp, synthetic construct
  misc_feature 1..20: note = 5' hIgHD HU2(h268)
  source 1..20: mol_type = other DNA
gcagtaaccctcaggaagca

SEQ ID NO: 80 - DNA, 31 bp, synthetic construct
  misc_feature 1..31: note = 3' hIgHD HU2 AgeI(h269)
  source 1..31: mol_type = other DNA
cttccaccggtacagccacaccaaggtcatc

SEQ ID NO: 81 - DNA, 31 bp, synthetic construct
  misc_feature 1..31: note = 5' hIgHD HD2 XhoI(h271)
  source 1..31: mol_type = other DNA
cttccctcgaggaacactgtcagctcccaca

SEQ ID NO: 82 - DNA, 19 bp, synthetic construct
  misc_feature 1..19: note = 3' hIgHD HD2(h272)
  source 1..19: mol_type = other DNA
agatcctccatgcgtgctg

SEQ ID NO: 83 - DNA, 20 bp, synthetic construct
  misc_feature 1..20: note = 5' hIgHD HU2 detect(h270)
  source 1..20: mol_type = other DNA
tctcctctcgtcgcctctac

SEQ ID NO: 84 - DNA, 21 bp, synthetic construct
  misc_feature 1..21: note = 3' ub pro-200
  source 1..21: mol_type = other DNA
ccagtgccctagagtcaccca

SEQ ID NO: 85 - DNA, 21 bp, synthetic construct
  misc_feature 1..21: note = 5' neo detect
  source 1..21: mol_type = other DNA
ctcccactcatgatctataga

SEQ ID NO: 86 - DNA, 20 bp, synthetic construct
  misc_feature 1..20: note = 3' hIgHD HD2 detect(h273)
  source 1..20: mol_type = other DNA
gggtgcttgggtcctgttag

SEQ ID NO: 87 - DNA, 23 bp, synthetic construct
  misc_feature 1..23: note = 5' D2-2 Cas9 DNA target
  source 1..23: mol_type = other DNA
aggtctggagctacaagcggtgg

SEQ ID NO: 88 - RNA, 42 nt, synthetic construct
  misc_feature 1..42: note = 5' D2-2 gRNA
  source 1..42: mol_type = other RNA
aggtctggagctacaagcgggttttagagctatgctgttttg

SEQ ID NO: 89 - DNA, 23 bp, synthetic construct
  misc_feature 1..23: note = 3' D2-2 Cas9 DNA target
  source 1..23: mol_type = other DNA
aggacaacagtgagggttacagg

SEQ ID NO: 90 - RNA, 42 nt, synthetic construct
  misc_feature 1..42: note = 3' D2-2 gRNA
  source 1..42: mol_type = other RNA
aggacaacagtgagggttacgttttagagctatgctgttttg

SEQ ID NO: 91 - DNA, 19 bp, synthetic construct
  misc_feature 1..19: note = 5' up detect D2-2(h274)
  source 1..19: mol_type = other DNA
gtcaaaggtggaggcagtg

SEQ ID NO: 92 - DNA, 21 bp, synthetic construct
  misc_feature 1..21: note = 3' cm up detect
  source 1..21: mol_type = other DNA
tccagctgaacggtctggtta

SEQ ID NO: 93 - DNA, 19 bp, synthetic construct
  misc_feature 1..19: note = D2-2seqF2
  source 1..19: mol_type = other DNA
agcgattcaacagctaacc

SEQ ID NO: 94 - DNA, 20 bp, synthetic construct
  misc_feature 1..20: note = 3' down detect D2-2(h275)
  source 1..20: mol_type = other DNA
ccagtagaagtaacgaccac

SEQ ID NO: 95 - DNA, 80 bp, synthetic construct
  misc_feature 1..80: note = JO-1
  source 1..80: mol_type = other DNA
ctccagacccccaagactgggacctgccttcctgccaccgcttgtagctccagacctccgtgcctcccccgaccacttac

SEQ ID NO: 96 - DNA, 19 bp, synthetic construct
  misc_feature 1..19: note = 5' up detect D2-2(h274)
  source 1..19: mol_type = other DNA
gtcaaaggtggaggcagtg

SEQ ID NO: 97 - DNA, 19 bp, synthetic construct
  misc_feature 1..19: note = D2-2seqR1
  source 1..19: mol_type = other DNA
cccgtgcctagatcaatgc

SEQ ID NO: 98 - DNA, 19 bp, synthetic construct
  misc_feature 1..19: note = D2-2seqF1
  source 1..19: mol_type = other DNA
aggcattgatctaggcacg

SEQ ID NO: 99 - DNA, 19 bp, synthetic construct
  misc_feature 1..19: note = D2-2seqR2
  source 1..19: mol_type = other DNA
ctgttgaatcgctgcaagc

SEQ ID NO: 100 - DNA, 23 bp, synthetic construct
  misc_feature 1..23: note = 5' D2-8 Cas9 DNA target
  source 1..23: mol_type = other DNA
acctgaagacgcccagtcaacgg

SEQ ID NO: 101 - RNA, 42 nt, synthetic construct
  misc_feature 1..42: note = 5' D2-8 crRNA
  source 1..42: mol_type = other RNA
acctgaagacgcccagtcaagttttagagctatgctgttttg

SEQ ID NO: 102 - DNA, 23 bp, synthetic construct
  misc_feature 1..23: note = 3' D2-8 Cas9 DNA target
  source 1..23: mol_type = other DNA
gccacaagcacaaaagtacaggg

SEQ ID NO: 103 - RNA, 42 nt, synthetic construct
  misc_feature 1..42: note = 3' D2-8 crRNA
  source 1..42: mol_type = other RNA
gccacaagcacaaaagtacagttttagagctatgctgttttg

SEQ ID NO: 104 - DNA, 19 bp, synthetic construct
  misc_feature 1..19: note = 5' up detect D2-8(h276)
  source 1..19: mol_type = other DNA
gccttacccaagtctttcc

SEQ ID NO: 105 - DNA, 21 bp, synthetic construct
  misc_feature 1..21: note = 3' cm up detect
  source 1..21: mol_type = other DNA
tccagctgaacggtctggtta

SEQ ID NO: 106 - DNA, 19 bp, synthetic construct
  misc_feature 1..19: note = D2-8seqF2
  source 1..19: mol_type = other DNA
tccaataagtcggttcggc

SEQ ID NO: 107 - DNA, 19 bp, synthetic construct
  misc_feature 1..19: note = 3' down detect D2-8(h277)
  source 1..19: mol_type = other DNA
gcagaagtaaccaccactg

SEQ ID NO: 108 - DNA, 80 bp, synthetic construct
  misc_feature 1..80: note = JO-2
  source 1..80: mol_type = other DNA
tcacaggcctctcctgggaagagacctgaagacgcccagtcaacggagtctaacaccaaacctccctggaggccgatggg

SEQ ID NO: 109 - DNA, 19 bp, synthetic construct
  misc_feature 1..19: note = 5' up detect D2-8(h276)
  source 1..19: mol_type = other DNA
gccttacccaagtctttcc

SEQ ID NO: 110 - DNA, 20 bp, synthetic construct
  misc_feature 1..20: note = D2-8seqR1
  source 1..20: mol_type = other DNA
gccctacttgtagttacgtg

SEQ ID NO: 111 - DNA, 19 bp, synthetic construct
  misc_feature 1..19: note = D2-8seqF1
  source 1..19: mol_type = other DNA
gcaaaatccgacacgtaac

SEQ ID NO: 112 - DNA, 20 bp, synthetic construct
  misc_feature 1..20: note = D2-8seqR2
  source 1..20: mol_type = other DNA
cgaaccgacttattggatgc

SEQ ID NO: 113 - DNA, 23 bp, synthetic construct
  misc_feature 1..23: note = 5' D2-8 Cas9 DNA target
  source 1..23: mol_type = other DNA
ggtggccccataacacacctagg

SEQ ID NO: 114 - RNA, 42 nt, synthetic construct
  misc_feature 1..42: note = 5' D2-8 crRNA
  source 1..42: mol_type = other RNA
ggtggccccataacacacctgttttagagctatgctgttttg

SEQ ID NO: 115 - DNA, 23 bp, synthetic construct
  misc_feature 1..23: note = 3' D2-8 Cas9 DNA target
  source 1..23: mol_type = other DNA
ggacaacagtagagggctacagg

SEQ ID NO: 116 - RNA, 42 nt, synthetic construct
  misc_feature 1..42: note = 3' D2-8 crRNA
  source 1..42: mol_type = other RNA
ggacaacagtagagggctacgttttagagctatgctgttttg

SEQ ID NO: 117 - DNA, 20 bp, synthetic construct
  misc_feature 1..20: note = 5' up detect D2-15(h278)
  source 1..20: mol_type = other DNA
gcactccctctaaagacaag

SEQ ID NO: 118 - DNA, 21 bp, synthetic construct
  misc_feature 1..21: note = 3' cm up detect
  source 1..21: mol_type = other DNA
tccagctgaacggtctggtta

SEQ ID NO: 119 - DNA, 19 bp, synthetic construct
  misc_feature 1..19: note = D2-15seqF2
  source 1..19: mol_type = other DNA
gtaaaaataccgccgctgg

SEQ ID NO: 120 - DNA, 19 bp, synthetic construct
  misc_feature 1..19: note = 3' down detect D2-15(h279)
  source 1..19: mol_type = other DNA
gcattttcctgttcttgcg

SEQ ID NO: 121 - DNA, 80 bp, synthetic construct
  misc_feature 1..80: note = JO-3
  source 1..80: mol_type = other DNA
gctgacatcccgagctcctcaatggtggccccataacacacctaggaaacataacacacccacagccccacctggaacag

SEQ ID NO: 122 - DNA, 20 bp, synthetic construct
  misc_feature 1..20: note = 5' up detect D2-15(h278)*
  source 1..20: mol_type = other DNA
gcactccctctaaagacaag

SEQ ID NO: 123 - DNA, 20 bp, synthetic construct
  misc_feature 1..20: note = D2-15seqR1
  source 1..20: mol_type = other DNA
ctgggagatattggtgcatc

SEQ ID NO: 124 - DNA, 19 bp, synthetic construct
  misc_feature 1..19: note = D2-15seqF1
  source 1..19: mol_type = other DNA
tgcaccaatatctcccagt

SEQ ID NO: 125 - DNA, 20 bp, synthetic construct
  misc_feature 1..20: note = D2-15seqR2
  source 1..20: mol_type = other DNA
cggcggtatttttactgacc

SEQ ID NO: 126 - DNA, 21 bp, synthetic construct
  misc_feature 1..21: note = 23D3.312-1
  source 1..21: mol_type = other DNA
tttttgtgcaccccttaatgg

SEQ ID NO: 127 - DNA, 22 bp, synthetic construct
  misc_feature 1..22: note = 23D3.312-1
  source 1..22: mol_type = other DNA
atgtggtattacgatttttgga

SEQ ID NO: 128 - DNA, 26 bp, synthetic construct
  misc_feature 1..26: note = 23D3.312-1
  source 1..26: mol_type = other DNA
tctgtgacactgtgggtataataacc

SEQ ID NO: 129 - DNA, 22 bp, synthetic construct
  misc_feature 1..22: note = 23D3.312-2
  source 1..22: mol_type = other DNA
cccacagtgtcacagagtccat

SEQ ID NO: 130 - DNA, 24 bp, synthetic construct
  misc_feature 1..24: note = 23D3.312-2
  source 1..24: mol_type = other DNA
caagatggctttccttctgcctcc

SEQ ID NO: 131 - DNA, 19 bp, synthetic construct
  misc_feature 1..19: note = 23D3.312-2
  source 1..19: mol_type = other DNA
tcccagctccaggacagag

SEQ ID NO: 132 - DNA, 24 bp, synthetic construct
  misc_feature 1..24: note = 23D3.312-3
  source 1..24: mol_type = other DNA
tgtcacagagtccatcaaaaacct

SEQ ID NO: 133 - DNA, 14 bp, synthetic construct
  misc_feature 1..14: note = 23D3.312-3
  source 1..14: mol_type = other DNA
caccaccccctctc

SEQ ID NO: 134 - DNA, 19 bp, synthetic construct
  misc_feature 1..19: note = 23D3.312-3
  source 1..19: mol_type = other DNA
cctgagaccctggcaagct

SEQ ID NO: 135 - DNA, 19 bp, synthetic construct
  misc_feature 1..19: note = Jxn DH2-2
  source 1..19: mol_type = other DNA
atggcgcttgcagcgattc

SEQ ID NO: 136 - DNA, 28 bp, synthetic construct
  misc_feature 1..28: note = Jxn DH2-2
  source 1..28: mol_type = other DNA
ccaatactaacgaggaaatgcaaaccca

SEQ ID NO: 137 - DNA, 21 bp, synthetic construct
  misc_feature 1..21: note = Jxn DH2-2
  source 1..21: mol_type = other DNA
accctcactgttgtccttctg

SEQ ID NO: 138 - DNA, 23 bp, synthetic construct
  misc_feature 1..23: note = Jxn DH2-8
  source 1..23: mol_type = other DNA
gcaaacgtccatctgaaggagaa

SEQ ID NO: 139 - DNA, 27 bp, synthetic construct
  misc_feature 1..27: note = Jxn DH2-8
  source 1..27: mol_type = other DNA
caaataaacgatggcaggctacacccg

SEQ ID NO: 140 - DNA, 22 bp, synthetic construct
  misc_feature 1..22: note = Jxn DH2-8
  source 1..22: mol_type = other DNA
gagttgccgaaccgacttattg

SEQ ID NO: 141 - DNA, 23 bp, synthetic construct
  misc_feature 1..23: note = Jxn DH2-15
  source 1..23: mol_type = other DNA
gcaatggtaggttcatgtccatc

SEQ ID NO: 142 - DNA, 20 bp, synthetic construct
  misc_feature 1..20: note = Jxn DH2-15
  source 1..20: mol_type = other DNA
accgccgctggtactccaat

SEQ ID NO: 143 - DNA, 19 bp, synthetic construct
  misc_feature 1..19: note = Jxn DH2-15
  source 1..19: mol_type = other DNA
ccctggctgtctgggtttg

SEQ ID NO: 144-145 - skipped (2 entries)

SEQ ID NO: 146 - DNA, 29 bp, synthetic construct
  misc_feature 1..29: note = Template switching oligo
  source 1..29: mol_type = other DNA
agcagtggtatcaacgcagagtacatggg

SEQ ID NO: 147 - DNA, 54 bp, synthetic construct
  misc_feature 1..54: note = 1st round PCR primers IgM Constant
  source 1..54: mol_type = other DNA
acactctttccctacacgacgctcttccgatctgggaagacatttgggaaggac

SEQ ID NO: 148 - DNA, 57 bp, synthetic construct
  misc_feature 1..57: note = 1st round PCR primers PE2-PIIA
  source 1..57: mol_type = other DNA
gtgactggagttcagacgtgtgctcttccgatctaagcagtggtatcaacgcagagt

SEQ ID NO: 149 - DNA, 68 bp, synthetic construct
  misc_feature 1..68: note = 2nd round PCR Primers
  source 1..68: mol_type = other DNA
  variation 30..35: note = n is a, c, g, or t
aatgatacggcgaccaccgagatctacacnnnnnnacactctttccctacacgacgctcttccgatct

SEQ ID NO: 150 - DNA, 64 bp, synthetic construct
  misc_feature 1..64: note = 2nd round PCR Primers
  source 1..64: mol_type = other DNA
  variation 25..30: note = n is a, c, g, or t
caagcagaagacggcatacgagatnnnnnngtgactggagttcagacgtgtgctcttccgatct

SEQ ID NO: 151 - DNA, 39 bp, synthetic construct
  misc_feature 1..39: note = 23-mer RSS from VH1-69
  source 1..39: mol_type = other DNA
cacagtgtgaaaacccacatcctgagagtgacacaaacc